European Patent Application EP 4 424 845 A1, published September 4, 2024. Title: METHOD, KIT AND CARTRIDGE FOR DETECTING NUCLEIC ACID MOLECULE. Applicant: Personal Genomics Taiwan, Inc. The sequence listing filed with the application follows.

SEQUENCE LISTING (6 sequences)

SEQ ID NO: 1 - DNA, 22 bp, synthetic construct
  source 1..22: mol_type = other DNA
ttggaacaggaagagaatcagc

SEQ ID NO: 2 - DNA, 22 bp, synthetic construct
  source 1..22: mol_type = other DNA
tgacaccaccaaaagaacatgg

SEQ ID NO: 3 - DNA, 25 bp, synthetic construct
  source 1..25: mol_type = other DNA
cagactcctacggggaggcagcagt

SEQ ID NO: 4 - DNA, 24 bp, synthetic construct
  source 1..24: mol_type = other DNA
acttaacccaacatctcacgacac

SEQ ID NO: 5 - DNA, 20 bp, synthetic construct
  source 1..20: mol_type = other DNA
ccaccgggactcagattctc

SEQ ID NO: 6 - DNA, 19 bp, synthetic construct
  source 1..19: mol_type = other DNA
tgtcgtccacgtagcccac